European Patent Specification EP 3 845 649 B1, published September 24, 2025. Title: Nucleic acid-drug complex and use thereof. Applicant: Industrial Technology Research Institute. The sequence listing filed with the application follows.

SEQUENCE LISTING (34 sequences)

SEQ ID NO: 1 - DNA, 30 bp, Artificial Sequence
  anti-PD-L1 aptamer
cacatcaactcattgatagacaatgcgtcc

SEQ ID NO: 2 - DNA, 35 bp, Artificial Sequence
  anti-PD-L1 aptamer
ccacatcaactcattgatagacaatgcgtccaccg

SEQ ID NO: 3 - DNA, 21 bp, Artificial Sequence
  anti-PD-L1 aptamer
actcattgatagacaatgcgt

SEQ ID NO: 4 - DNA, 21 bp, Artificial Sequence
  anti-PD-L1 aptamer
agcgattgatagacaatcgct

SEQ ID NO: 5 - DNA, 26 bp, Artificial Sequence
  anti-PD-L1 aptamer
atgaactcattcatacacaatgcgtg

SEQ ID NO: 6 - DNA, 32 bp, Artificial Sequence
  anti-PD-L1 aptamer
gttgttttttcactcattgatagacaatgcgt

SEQ ID NO: 7 - DNA, 30 bp, Artificial Sequence
  anti-PD-L1 aptamer
agttatgctttccccctctttgatagacaa

SEQ ID NO: 8 - DNA, 31 bp, Artificial Sequence
  anti-PD-L1 aptamer
gaacaaaggtattagacatcttgatagacaa

SEQ ID NO: 9 - DNA, 30 bp, Artificial Sequence
  anti-PD-L1 aptamer
actcattgatagacaatgcgtgcccgcagc

SEQ ID NO: 10 - DNA, 30 bp, Artificial Sequence
  CpG sequence
  misc_difference (1)..(29): phosphorothioate bond
tcgaacgttcgaacgttcgaacgttcgaat

SEQ ID NO: 11 - DNA, 20 bp, mouse
  misc_difference (1)..(19): phosphorothioate bond
tccatgacgttcctgacgtt

SEQ ID NO: 12 - DNA, 24 bp, Homo sapiens
  misc_difference (1)..(23): phosphorothioate bond
tcgtcgttttgtcgttttgtcgtt

SEQ ID NO: 13 - DNA, 20 bp, mouse
  misc_difference (1)..(2): phosphorothioate bond
  misc_difference (15)..(19): phosphorothioate bond
ggggtcaacgttgagggggg

SEQ ID NO: 14 - DNA, 20 bp, mouse
  misc_difference (1)..(19): phosphorothioate bond
tccatgacgttcctgatgct

SEQ ID NO: 15 - DNA, 22 bp, Bovine
  misc_difference (1)..(21): phosphorothioate bond
tcgtcgttgtcgttttgtcgtt

SEQ ID NO: 16 - DNA, 23 bp, Homo sapiens
  misc_difference (1)..(22): phosphorothioate bond
tcgacgttcgtcgttcgtcgttc

SEQ ID NO: 17 - DNA, 22 bp, Homo sapiens
  misc_difference (1)..(21): phosphorothioate bond
tgactgtgaacgttcgagatga

SEQ ID NO: 18 - DNA, 26 bp, unknown
  multi-species
  misc_difference (1)..(25): phosphorothioate bond
tcgcgacgttcgcccgacgttcggta

SEQ ID NO: 19 - DNA, 29 bp, unknown
  multi-species
  misc_difference (1)..(28): phosphorothioate bond
tcgcgaacgttcgccgcgttcgaacgcgg

SEQ ID NO: 20 - DNA, 21 bp, Homo sapiens
  misc_difference (1)..(20): phosphorothioate bond
tcgtcgaacgttcgagatgat

SEQ ID NO: 21 - DNA, 25 bp, Homo sapiens
  misc_difference (1)..(24): phosphorothioate bond
tcgaacgttcgaacgttcgaacgtt

SEQ ID NO: 22 - DNA, 30 bp, Artificial Sequence
  CpG sequence
  misc_difference (1)..(29): phosphorothioate bond
tcgaacgttcgaacgtcgaacgttcgaacg

SEQ ID NO: 23 - DNA, 30 bp, Artificial Sequence
  CpG sequence
  misc_difference (1)..(29): phosphorothioate bond
ttcgaacgttcgaatttcgaacgttcgaat

SEQ ID NO: 24 - DNA, 45 bp, Artificial Sequence
  anti-PD-L1 aptamer
acgggccacatcaactcattgatagacaatgcgtccactgcccgt

SEQ ID NO: 25 - DNA, 60 bp, Artificial Sequence
  anti-PD-L1 aptamer-CpG sequence
  misc_difference (1)..(29): phosphorothioate bond
tcgaacgttcgaacgttcgaacgttcgaatcacatcaactcattgatagacaatgcgtcc

SEQ ID NO: 26 - DNA, 60 bp, Artificial Sequence; identical to SEQ ID NO: 25
  anti-PD-L1 aptamer-CpG sequence
  misc_difference (2)..(2): phosphorothioate bond
  misc_difference (6)..(6): phosphorothioate bond
  misc_difference (10)..(10): phosphorothioate bond
  misc_difference (14)..(14): phosphorothioate bond
  misc_difference (18)..(18): phosphorothioate bond
  misc_difference (22)..(22): phosphorothioate bond
  misc_difference (26)..(26): phosphorothioate bond

SEQ ID NO: 27 - DNA, 60 bp, Artificial Sequence
  anti-PD-L1 aptamer-CpG sequence
  misc_difference (31)..(59): phosphorothioate bond
cacatcaactcattgatagacaatgcgtcctcgaacgttcgaacgttcgaacgttcgaat

SEQ ID NO: 28 - DNA, 60 bp, Artificial Sequence
  anti-PD-L1 aptamer-CpG sequence
  misc_difference (33)..(33): phosphorothioate bond
  misc_difference (37)..(37): phosphorothioate bond
  misc_difference (41)..(41): phosphorothioate bond
  misc_difference (45)..(45): phosphorothioate bond
  misc_difference (49)..(49): phosphorothioate bond
  misc_difference (53)..(53): phosphorothioate bond
  misc_difference (57)..(59): phosphorothioate bond
cacatcaactcattgatagacaatgcgtccttcgaacgttcgaacgttcgaacgttcgaa

SEQ ID NO: 29 - DNA, 60 bp, Artificial Sequence
  anti-PD-L1 aptamer-CpG sequence
  misc_difference (1)..(14): phosphorothioate bond
  misc_difference (46)..(59): phosphorothioate bond
tcgaacgttcgaacgcacatcaactcattgatagacaatgcgtccttcgaacgttcgaat

SEQ ID NO: 30 - DNA, 67 bp, Artificial Sequence
  anti-PD-L1 aptamer-CpG sequence
  misc_difference (1)..(2): phosphorothioate bond
  misc_difference (66)..(66): phosphorothioate bond
tttcgaacgttcgaacgccacatcaactcattgatagacaatgcgtccaccgttcgaacgttcgatt

SEQ ID NO: 31 - DNA, 51 bp, Artificial Sequence
  anti-PD-L1 aptamer-CpG sequence
  misc_difference (1)..(14): phosphorothioate bond
  misc_difference (37)..(50): phosphorothioate bond
tcgaacgttcgaacgactcattgatagacaatgcgtttcgaacgttcgaat

SEQ ID NO: 32 - DNA, 51 bp, Artificial Sequence
  anti-PD-L1 aptamer-CpG sequence
  misc_difference (1)..(14): phosphorothioate bond
  misc_difference (37)..(50): phosphorothioate bond
tcgaacgttcgaacgactcattgatagacaatgcgttcgaacgttcgaacg

SEQ ID NO: 33 - DNA, 50 bp, Artificial Sequence
  anti-PD-L1 aptamer-CpG sequence
  misc_difference (1)..(13): phosphorothioate bond
  misc_difference (36)..(49): phosphorothioate bond
tcgaacgttcgaatactcattgatagacaatgcgtttcgaacgttcgaat

SEQ ID NO: 34 - DNA, 60 bp, Artificial Sequence
  anti-PD-L1 aptamer-CpG sequence
  misc_difference (1)..(14): phosphorothioate bond
  misc_difference (46)..(59): phosphorothioate bond
tcgaacgttcgaacgagttatgctttccccctctttgatagacaattcgaacgttcgaat